European Patent Specification EP 3 687 562 B1, published March 19, 2025. Title: TREATMENT OF INFLAMMATORY CONDITIONS BY DELIVERY OF INTERLEUKIN-1 RECEPTOR ANTAGONIST FUSION PROTEIN. Applicant: Regeneron Pharmaceuticals, Inc. Application Filing herewith. The sequence listing filed with the application follows.

SEQUENCE LISTING (5 sequences)

SEQ ID NO: 1 - protein, 880 aa, Artificial Sequence
  Synthetic Polypeptide
SERCDDWGLDTMRQIQVFEDEPARIKCPLFEHFLKFNYSTAHSAGLTLIWYWTRQDRDLEEPINFRLPENRISKEKDVLWFRPTLLNDTGNYTCMLRNTTYCSKVAFPLEVVQKDSCFNSPMKLPVHKLYIEYGIQRITCPNVDGYFPSSVKPTITWYMGCYKIQNFNNVIPEGMNLSFLIALISNNGNYTCVVTYPENGRTFHLTRTLTVKVVGSPKNAVPPVIHSPNDHVVYEKEPGEELLIPCTVYFSFLMDSRNEVWWTIDGKKPDDITIDVTINESISHSRTEDETRTQILSIKKVTSEDLKRSYVCHARSAKGEVAKAAKVKQKVPAPRYTVEKCKEREEKIILVSSANEIDVRPCPLNPNEHKGTITWYKDDSKTPVSTEQASRIHQHKEKLWFVPAKVEDSGHYYCVVRNSSYCLRIKISAKFVENEPNLCYNAQAIFKQKLPVAGDGGLVCPYMEFFKNENNELPKLQWYKDCKPLLLDNIHFSGVKDRLIVMNVAEKHRGNYTCHASYTYLGKQYPITRVIEFITLEENKPTRPVIVSPANETMEVDLGSQIQLICNVTGQLSDIAYWKWNGSVIDEDDPVLGEDYYSVENPANKRRSTLITVLNISEIESRFYKHPFTCFAKNTHGIDAAYIQLIYPVTNSGDKTHTCPPCPAPELLGGPSVFLFPPKPKDTLMISRTPEVTCVVVDVSHEDPEVKFNWYVDGVEVHNAKTKPREEQYNSTYRVVSVLTVLHQDWLNGKEYKCKVSNKALPAPIEKTISKAKGQPREPQVYTLPPSRDELTKNQVSLTCLVKGFYPSDIAVEWESNGQPENNYKTTPPVLDSDGSFFLYSKLTVDKSRWQQGNVFSCSVMHEALHNHYTQKSLSLSPGK

SEQ ID NO: 2 - protein, 900 aa, Artificial Sequence
  Synthetic Polypeptide
MVLLWCVVSLYFYGILQSDASERCDDWGLDTMRQIQVFEDEPARIKCPLFEHFLKFNYSTAHSAGLTLIWYWTRQDRDLEEPINFRLPENRISKEKDVLWFRPTLLNDTGNYTCMLRNTTYCSKVAFPLEVVQKDSCFNSPMKLPVHKLYIEYGIQRITCPNVDGYFPSSVKPTITWYMGCYKIQNFNNVIPEGMNLSFLIALISNNGNYTCVVTYPENGRTFHLTRTLTVKVVGSPKNAVPPVIHSPNDHVVYEKEPGEELLIPCTVYFSFLMDSRNEVWWTIDGKKPDDITIDVTINESISHSRTEDETRTQILSIKKVTSEDLKRSYVCHARSAKGEVAKAAKVKQKVPAPRYTVEKCKEREEKIILVSSANEIDVRPCPLNPNEHKGTITWYKDDSKTPVSTEQASRIHQHKEKLWFVPAKVEDSGHYYCVVRNSSYCLRIKISAKFVENEPNLCYNAQAIFKQKLPVAGDGGLVCPYMEFFKNENNELPKLQWYKDCKPLLLDNIHFSGVKDRLIVMNVAEKHRGNYTCHASYTYLGKQYPITRVIEFITLEENKPTRPVIVSPANETMEVDLGSQIQLICNVTGQLSDIAYWKWNGSVIDEDDPVLGEDYYSVENPANKRRSTLITVLNISEIESRFYKHPFTCFAKNTHGIDAAYIQLIYPVTNSGDKTHTCPPCPAPELLGGPSVFLFPPKPKDTLMISRTPEVTCVVVDVSHEDPEVKFNWYVDGVEVHNAKTKPREEQYNSTYRVVSVLTVLHQDWLNGKEYKCKVSNKALPAPIEKTISKAKGQPREPQVYTLPPSRDELTKNQVSLTCLVKGFYPSDIAVEWESNGQPENNYKTTPPVLDSDGSFFLYSKLTVDKSRWQQGNVFSCSVMHEALHNHYTQKSLSLSPGK

SEQ ID NO: 3 - protein, 339 aa, Artificial Sequence
  Synthetic Polypeptide
SERCDDWGLDTMRQIQVFEDEPARIKCPLFEHFLKFNYSTAHSAGLTLIWYWTRQDRDLEEPINFRLPENRISKEKDVLWFRPTLLNDTGNYTCMLRNTTYCSKVAFPLEVVQKDSCFNSPMKLPVHKLYIEYGIQRITCPNVDGYFPSSVKPTITWYMGCYKIQNFNNVIPEGMNLSFLIALISNNGNYTCVVTYPENGRTFHLTRTLTVKVVGSPKNAVPPVIHSPNDHVVYEKEPGEELLIPCTVYFSFLMDSRNEVWWTIDGKKPDDITIDVTINESISHSRTEDETRTQILSIKKVTSEDLKRSYVCHARSAKGEVAKAAKVKQKVPAPRYTVE

SEQ ID NO: 4 - protein, 312 aa, Artificial Sequence
  Synthetic Polypeptide
KCKEREEKIILVSSANEIDVRPCPLNPNEHKGTITWYKDDSKTPVSTEQASRIHQHKEKLWFVPAKVEDSGHYYCVVRNSSYCLRIKISAKFVENEPNLCYNAQAIFKQKLPVAGDGGLVCPYMEFFKNENNELPKLQWYKDCKPLLLDNIHFSGVKDRLIVMNVAEKHRGNYTCHASYTYLGKQYPITRVIEFITLEENKPTRPVIVSPANETMEVDLGSQIQLICNVTGQLSDIAYWKWNGSVIDEDDPVLGEDYYSVENPANKRRSTLITVLNISEIESRFYKHPFTCFAKNTHGIDAAYIQLIYPVTN

SEQ ID NO: 5 - protein, 227 aa, Artificial Sequence
  Synthetic Polypeptide
DKTHTCPPCPAPELLGGPSVFLFPPKPKDTLMISRTPEVTCVVVDVSHEDPEVKFNWYVDGVEVHNAKTKPREEQYNSTYRVVSVLTVLHQDWLNGKEYKCKVSNKALPAPIEKTISKAKGQPREPQVYTLPPSRDELTKNQVSLTCLVKGFYPSDIAVEWESNGQPENNYKTTPPVLDSDGSFFLYSKLTVDKSRWQQGNVFSCSVMHEALHNHYTQKSLSLSPGK